European Patent Application EP 4 549 581 A1, published May 7, 2025. Title: HIGHLY SENSITIVE METHODS FOR ACCURATE PARALLEL QUANTIFICATION OF NUCLEIC ACIDS. Applicant: Genomill Health Oy. The sequence listing filed with the application follows.

SEQUENCE LISTING (31 sequences)

SEQ ID NO: 1 - DNA, 31 bp, synthetic construct
  source 1..31: mol_type = other DNA
ggggcccgccgtcgatcggagccgttaggat

SEQ ID NO: 2 - DNA, 31 bp, synthetic construct
  source 1..31: mol_type = other DNA
ttaaggtgccgtcgatcggagccgacgtacg

SEQ ID NO: 3 - DNA, 31 bp, synthetic construct; identical to SEQ ID NO: 2
  source 1..31: mol_type = other DNA

SEQ ID NO: 4 - DNA, 31 bp, synthetic construct
  source 1..31: mol_type = other DNA
tataatagaggtcgtgcagtcacgacccggt

SEQ ID NO: 5 - DNA, 31 bp, synthetic construct
  source 1..31: mol_type = other DNA
accaggtgccgtcgatcggagccgacccggt

SEQ ID NO: 6 - DNA, 31 bp, synthetic construct
  source 1..31: mol_type = other DNA
gggccgggaggtcgtgcagtcacgttaggat

SEQ ID NO: 7 - DNA, 31 bp, synthetic construct
  source 1..31: mol_type = other DNA
tccaggtgagtcgatccgtcacgtacgtacg

SEQ ID NO: 8 - DNA, 31 bp, synthetic construct
  source 1..31: mol_type = other DNA
aaaattttagcgtacgtcgtacgtttaggat

SEQ ID NO: 9 - DNA, 31 bp, synthetic construct; identical to SEQ ID NO: 4
  source 1..31: mol_type = other DNA

SEQ ID NO: 10 - DNA, 31 bp, synthetic construct
  source 1..31: mol_type = other DNA
aggaccttgagtcgatccgcacgtacccggt

SEQ ID NO: 11 - DNA, 31 bp, synthetic construct
  source 1..31: mol_type = other DNA
agcgaccgaggtcgtgcagtcacgacgtacg

SEQ ID NO: 12 - DNA, 31 bp, synthetic construct; identical to SEQ ID NO: 4
  source 1..31: mol_type = other DNA

SEQ ID NO: 13 - DNA, 31 bp, synthetic construct
  source 1..31: mol_type = other DNA
ggaaaaagccgtcgatcggagccgttaggat

SEQ ID NO: 14 - DNA, 31 bp, synthetic construct
  source 1..31: mol_type = other DNA
atatacagaggtcgtgcagtcacgttaggat

SEQ ID NO: 15 - DNA, 31 bp, synthetic construct
  source 1..31: mol_type = other DNA
gagagccgaggtcgtgcagtcacgacccggt

SEQ ID NO: 16 - DNA, 31 bp, synthetic construct
  source 1..31: mol_type = other DNA
cgcacgcgaggtcgtgcagtcacgacgtacg

SEQ ID NO: 17 - DNA, 31 bp, synthetic construct
  source 1..31: mol_type = other DNA
attacaagccgtcgatcggagccgacccggt

SEQ ID NO: 18 - DNA, 31 bp, synthetic construct; identical to SEQ ID NO: 4
  source 1..31: mol_type = other DNA

SEQ ID NO: 19 - DNA, 31 bp, synthetic construct
  source 1..31: mol_type = other DNA
gggcaattagcgtacgtcgtacgtacgtacg

SEQ ID NO: 20 - DNA, 31 bp, synthetic construct
  source 1..31: mol_type = other DNA
tatgcgagccgtcgatcggagccgacgtacg

SEQ ID NO: 21 - DNA, 31 bp, synthetic construct; identical to SEQ ID NO: 10
  source 1..31: mol_type = other DNA

SEQ ID NO: 22 - DNA, 31 bp, synthetic construct; identical to SEQ ID NO: 17
  source 1..31: mol_type = other DNA

SEQ ID NO: 23 - DNA, 31 bp, synthetic construct
  source 1..31: mol_type = other DNA
gaagaattagcgtacgtcgtacgtttaggat

SEQ ID NO: 24 - DNA, 31 bp, synthetic construct; identical to SEQ ID NO: 19
  source 1..31: mol_type = other DNA

SEQ ID NO: 25 - DNA, 31 bp, synthetic construct; identical to SEQ ID NO: 19
  source 1..31: mol_type = other DNA

SEQ ID NO: 26 - DNA, 31 bp, synthetic construct
  source 1..31: mol_type = other DNA
gagcacttagcgtacgtcgtacgtacccggt

SEQ ID NO: 27 - DNA, 31 bp, synthetic construct
  source 1..31: mol_type = other DNA
aaaggggcgagtcgatccgcacgtttaggat

SEQ ID NO: 28 - DNA, 31 bp, synthetic construct
  source 1..31: mol_type = other DNA
agcgcgcgccgtcgatcggagccgttaggat

SEQ ID NO: 29 - DNA, 40 bp, synthetic construct
  source 1..40: mol_type = other DNA
cgacgacgacagaaccagatacacgacgtacgcacgacat

SEQ ID NO: 30 - DNA, 59 bp, synthetic construct
  source 1..59: mol_type = other DNA
ggttctgtcgtcgtcggacacgacgctccgctnnnnnnnnnnagctgagcgtattcgat

SEQ ID NO: 31 - DNA, 68 bp, synthetic construct
  source 1..68: mol_type = other DNA
ctggatcgtcgtatgctnnnnnnnnnngatcgacccattggagaagatgatgtcgtgcggtacgtcgt